European Patent Application EP 4 321 169 A1, published February 14, 2024. Title: Peptides for inhibiting angiogenesis and the use thereof. Applicant: Seoul National University Hospital. The sequence listing filed with the application follows.

SEQUENCE LISTING (21 sequences)

SEQ ID NO: 1 - protein, 20 aa, Artificial Sequence
  peptide 1
NRPEVTYPCSCEVKGEEDNS

SEQ ID NO: 2 - protein, 20 aa, Artificial Sequence
  peptide 2
NRPEVTAPASCEVKGEEDNS

SEQ ID NO: 3 - protein, 20 aa, Artificial Sequence
  peptide 3
NRPEVTYPCSCEVKGAAANS

SEQ ID NO: 4 - protein, 20 aa, Artificial Sequence
  peptide 4
NRPEVTAPASCEVKGAAANS

SEQ ID NO: 5 - protein, 20 aa, Artificial Sequence
  peptide 5
AAAAAAYPCAAAAAAEEDAA

SEQ ID NO: 6 - protein, 20 aa, Artificial Sequence
  peptide 6
AAAAAAAAAAAAAAAEEDAA

SEQ ID NO: 7 - protein, 20 aa, Artificial Sequence
  peptide 7
AAAAAAYPCAAAAAAAAAAA

SEQ ID NO: 8 - protein, 15 aa, Artificial Sequence
  peptide 8
VKCCGWVSFYNWTDN

SEQ ID NO: 9 - protein, 13 aa, Artificial Sequence
  peptide 9
SFYNWTDNAELMN

SEQ ID NO: 10 - protein, 16 aa, Artificial Sequence
  peptide 10
AELMNRPEVTYPCSCE

SEQ ID NO: 11 - protein, 21 aa, Artificial Sequence
  peptide 11
YPCSCEVKGEEDNSLSVRKGF

SEQ ID NO: 12 - protein, 26 aa, Artificial Sequence
  peptide 12
GFCEAPGNRTQSGNHPEDWPVYQEGC

SEQ ID NO: 13 - protein, 17 aa, Artificial Sequence
  peptide 13
YPCSCEVKGEEDNSLSV

SEQ ID NO: 14 - protein, 15 aa, Artificial Sequence
  peptide 14
RKGFCEAPGNRTQSG

SEQ ID NO: 15 - protein, 13 aa, Artificial Sequence
  peptide 15
NHPEDWPVYQEGC

SEQ ID NO: 16 - protein, 6 aa, Artificial Sequence
  Binding motif 1
AXAHTG

SEQ ID NO: 17 - protein, 5 aa, Artificial Sequence
  Binding motif 2
QLEXV

SEQ ID NO: 18 - protein, 7 aa, Artificial Sequence
  Binding motif 3
IYIXXXD

SEQ ID NO: 19 - protein, 5 aa, Artificial Sequence
  Binding motif 4
NNEXS

SEQ ID NO: 20 - protein, 11 aa, Artificial Sequence
  Binding motif 5
KDXGXYXCXXR

SEQ ID NO: 21 - protein, 9 aa, Artificial Sequence
  Binding motif 6
EEDXGXYTI